European Patent Application EP 4 177 346 A2, published May 10, 2023. Title: COMPOSITIONS AND METHODS OF IMPROVING SPECIFICITY IN GENOMIC ENGINEERING USING RNA-GUIDED ENDONUCLEASES. Applicant: DUKE UNIVERSITY. Application PCT/US2016/048798. The sequence listing filed with the application follows.

SEQUENCE LISTING (348 sequences)

SEQ ID NO: 1 - protein, 1368 aa, Streptococcus pyogenes
MDKKYSIGLAIGTNSVGWAVITDEYKVPSKKFKVLGNTDRHSIKKNLIGALLFDSGETAEATRLKRTARRRYTRRKNRICYLQEIFSNEMAKVDDSFFHRLEESFLVEEDKKHERHPIFGNIVDEVAYHEKYPTIYHLRKKLVDSTDKADLRLIYLALAHMIKFRGHFLIEGDLNPDNSDVDKLFIQLVQTYNQLFEENPINASGVDAKAILSARLSKSRRLENLIAQLPGEKKNGLFGNLIALSLGLTPNFKSNFDLAEDAKLQLSKDTYDDDLDNLLAQIGDQYADLFLAAKNLSDAILLSDILRVNTEITKAPLSASMIKRYDEHHQDLTLLKALVRQQLPEKYKEIFFDQSKNGYAGYIDGGASQEEFYKFIKPILEKMDGTEELLVKLNREDLLRKQRTFDNGSIPHQIHLGELHAILRRQEDFYPFLKDNREKIEKILTFRIPYYVGPLARGNSRFAWMTRKSEETITPWNFEEVVDKGASAQSFIERMTNFDKNLPNEKVLPKHSLLYEYFTVYNELTKVKYVTEGMRKPAFLSGEQKKAIVDLLFKTNRKVTVKQLKEDYFKKIECFDSVEISGVEDRFNASLGTYHDLLKIIKDKDFLDNEENEDILEDIVLTLTLFEDREMIEERLKTYAHLFDDKVMKQLKRRRYTGWGRLSRKLINGIRDKQSGKTILDFLKSDGFANRNFMQLIHDDSLTFKEDIQKAQVSGQGDSLHEHIANLAGSPAIKKGILQTVKVVDELVKVMGRHKPENIVIEMARENQTTQKGQKNSRERMKRIEEGIKELGSQILKEHPVENTQLQNEKLYLYYLQNGRDMYVDQELDINRLSDYDVDAIVPQSFLKDDSIDNKVLTRSDKNRGKSDNVPSEEVVKKMKNYWRQLLNAKLITQRKFDNLTKAERGGLSELDKAGFIKRQLVETRQITKHVAQILDSRMNTKYDENDKLIREVKVITLKSKLVSDFRKDFQFYKVREINNYHHAHDAYLNAVVGTALIKKYPKLESEFVYGDYKVYDVRKMIAKSEQEIGKATAKYFFYSNIMNFFKTEITLANGEIRKRPLIETNGETGEIVWDKGRDFATVRKVLSMPQVNIVKKTEVQTGGFSKESILPKRNSDKLIARKKDWDPKKYGGFDSPTVAYSVLVVAKVEKGKSKKLKSVKELLGITIMERSSFEKNPIDFLEAKGYKEVKKDLIIKLPKYSLFELENGRKRMLASAGELQKGNELALPSKYVNFLYLASHYEKLKGSPEDNEQKQLFVEQHKHYLDEIIEQISEFSKRVILADANLDKVLSAYNKHRDKPIREQAENIIHLFTLTNLGAPAAFKYFDTTIDRKRYTSTKEVLDATLIHQSITGLYETRIDLSQLGGD

SEQ ID NO: 2 - protein, 2048 aa, Artificial Sequence
  Description of Artificial Sequence: Synthetic polypeptide
MDYKDHDGDYKDHDIDYKDDDDKMAPKKKRKVGRGMDKKYSIGLAIGTNSVGWAVITDEYKVPSKKFKVLGNTDRHSIKKNLIGALLFDSGETAEATRLKRTARRRYTRRKNRICYLQEIFSNEMAKVDDSFFHRLEESFLVEEDKKHERHPIFGNIVDEVAYHEKYPTIYHLRKKLVDSTDKADLRLIYLALAHMIKFRGHFLIEGDLNPDNSDVDKLFIQLVQTYNQLFEENPINASGVDAKAILSARLSKSRRLENLIAQLPGEKKNGLFGNLIALSLGLTPNFKSNFDLAEDAKLQLSKDTYDDDLDNLLAQIGDQYADLFLAAKNLSDAILLSDILRVNTEITKAPLSASMIKRYDEHHQDLTLLKALVRQQLPEKYKEIFFDQSKNGYAGYIDGGASQEEFYKFIKPILEKMDGTEELLVKLNREDLLRKQRTFDNGSIPHQIHLGELHAILRRQEDFYPFLKDNREKIEKILTFRIPYYVGPLARGNSRFAWMTRKSEETITPWNFEEVVDKGASAQSFIERMTNFDKNLPNEKVLPKHSLLYEYFTVYNELTKVKYVTEGMRKPAFLSGEQKKAIVDLLFKTNRKVTVKQLKEDYFKKIECFDSVEISGVEDRFNASLGTYHDLLKIIKDKDFLDNEENEDILEDIVLTLTLFEDREMIEERLKTYAHLFDDKVMKQLKRRRYTGWGRLSRKLINGIRDKQSGKTILDFLKSDGFANRNFMQLIHDDSLTFKEDIQKAQVSGQGDSLHEHIANLAGSPAIKKGILQTVKVVDELVKVMGRHKPENIVIEMARENQTTQKGQKNSRERMKRIEEGIKELGSQILKEHPVENTQLQNEKLYLYYLQNGRDMYVDQELDINRLSDYDVDAIVPQSFLKDDSIDNKVLTRSDKNRGKSDNVPSEEVVKKMKNYWRQLLNAKLITQRKFDNLTKAERGGLSELDKAGFIKRQLVETRQITKHVAQILDSRMNTKYDENDKLIREVKVITLKSKLVSDFRKDFQFYKVREINNYHHAHDAYLNAVVGTALIKKYPKLESEFVYGDYKVYDVRKMIAKSEQEIGKATAKYFFYSNIMNFFKTEITLANGEIRKRPLIETNGETGEIVWDKGRDFATVRKVLSMPQVNIVKKTEVQTGGFSKESILPKRNSDKLIARKKDWDPKKYGGFDSPTVAYSVLVVAKVEKGKSKKLKSVKELLGITIMERSSFEKNPIDFLEAKGYKEVKKDLIIKLPKYSLFELENGRKRMLASAGELQKGNELALPSKYVNFLYLASHYEKLKGSPEDNEQKQLFVEQHKHYLDEIIEQISEFSKRVILADANLDKVLSAYNKHRDKPIREQAENIIHLFTLTNLGAPAAFKYFDTTIDRKRYTSTKEVLDATLIHQSITGLYETRIDLSQLGGDPIAGSKASPKKKRKVGRAIFKPEELRQALMPTLEALYRQDPESLPFRQPVDPQLLGIPDYFDIVKSPMDLSTIKRKLDTGQYQEPWQYVDDIWLMFNNAWLYNRKTSRVYKYCSKLSEVFEQEIDPVMQSLGYCCGRKLEFSPQTLCCYGKQLCTIPRDATYYSYQNRYHFCEKCFNEIQGESVSLGDDPSQPQTTINKEQFSKRKNDTLDPELFVECTECGRKMHQICVLHHEIIWPAGFVCDGCLKKSARTRKENKFSAKRLPSTRLGTFLENRVNDFLRRQNHPESGEVTVRVVHASDKTVEVKPGMKARFVDSGEMAESFPYRTKALFAFEEIDGVDLCFFGMHVQEYGSDCPPPNQRRVYISYLDSVHFFRPKCLRTAVYHEILIGYLEYVKKLGYTTGHIWACPPSEGDDYIFHCHPPDQKIPKPKRLQEWYKKMLDKAVSERIVHDYKDIFKQATEDRLTSAKELPYFEGDFWPNVLEESIKELEQEEEERKREENTSNESTDVTKGDSKNAKKKNNKKTSKNKSSLSRGNKKKPGMPNVSNDLSQKLYATMEKHKEVFFVIRLIAGPAANSLPPIVDPDPLIPCDLMDGRDAFLTLARDKHLEFSSLRRAQWSTMCMLVELHTQSQDYPYDVPDYAS

SEQ ID NO: 3 - protein, 1521 aa, Artificial Sequence
  Description of Artificial Sequence: Synthetic polypeptide
MDYKDHDGDYKDHDIDYKDDDDKMAPKKKRKVGRGMDKKYSIGLAIGTNSVGWAVITDEYKVPSKKFKVLGNTDRHSIKKNLIGALLFDSGETAEATRLKRTARRRYTRRKNRICYLQEIFSNEMAKVDDSFFHRLEESFLVEEDKKHERHPIFGNIVDEVAYHEKYPTIYHLRKKLVDSTDKADLRLIYLALAHMIKFRGHFLIEGDLNPDNSDVDKLFIQLVQTYNQLFEENPINASGVDAKAILSARLSKSRRLENLIAQLPGEKKNGLFGNLIALSLGLTPNFKSNFDLAEDAKLQLSKDTYDDDLDNLLAQIGDQYADLFLAAKNLSDAILLSDILRVNTEITKAPLSASMIKRYDEHHQDLTLLKALVRQQLPEKYKEIFFDQSKNGYAGYIDGGASQEEFYKFIKPILEKMDGTEELLVKLNREDLLRKQRTFDNGSIPHQIHLGELHAILRRQEDFYPFLKDNREKIEKILTFRIPYYVGPLARGNSRFAWMTRKSEETITPWNFEEVVDKGASAQSFIERMTNFDKNLPNEKVLPKHSLLYEYFTVYNELTKVKYVTEGMRKPAFLSGEQKKAIVDLLFKTNRKVTVKQLKEDYFKKIECFDSVEISGVEDRFNASLGTYHDLLKIIKDKDFLDNEENEDILEDIVLTLTLFEDREMIEERLKTYAHLFDDKVMKQLKRRRYTGWGRLSRKLINGIRDKQSGKTILDFLKSDGFANRNFMQLIHDDSLTFKEDIQKAQVSGQGDSLHEHIANLAGSPAIKKGILQTVKVVDELVKVMGRHKPENIVIEMARENQTTQKGQKNSRERMKRIEEGIKELGSQILKEHPVENTQLQNEKLYLYYLQNGRDMYVDQELDINRLSDYDVDAIVPQSFLKDDSIDNKVLTRSDKNRGKSDNVPSEEVVKKMKNYWRQLLNAKLITQRKFDNLTKAERGGLSELDKAGFIKRQLVETRQITKHVAQILDSRMNTKYDENDKLIREVKVITLKSKLVSDFRKDFQFYKVREINNYHHAHDAYLNAVVGTALIKKYPKLESEFVYGDYKVYDVRKMIAKSEQEIGKATAKYFFYSNIMNFFKTEITLANGEIRKRPLIETNGETGEIVWDKGRDFATVRKVLSMPQVNIVKKTEVQTGGFSKESILPKRNSDKLIARKKDWDPKKYGGFDSPTVAYSVLVVAKVEKGKSKKLKSVKELLGITIMERSSFEKNPIDFLEAKGYKEVKKDLIIKLPKYSLFELENGRKRMLASAGELQKGNELALPSKYVNFLYLASHYEKLKGSPEDNEQKQLFVEQHKHYLDEIIEQISEFSKRVILADANLDKVLSAYNKHRDKPIREQAENIIHLFTLTNLGAPAAFKYFDTTIDRKRYTSTKEVLDATLIHQSITGLYETRIDLSQLGGDSRADPKKKRKVASDAKSLTAWSRTLVTFKDVFVDFTREEWKLLDTAQQILYRNVMLENYKNLVSLGYQLTKPDVILRLEKGEEPWLVEREIHQETHPDSETAFEIKSSVPKKKRKVAS

SEQ ID NO: 4 - protein, 617 aa, Artificial Sequence
  Description of Artificial Sequence: Synthetic polypeptide
YKVYDVRKMIAKSEQEIGKATAKYFFYSNIMNFFKTEITLANGEIRKRPLIETNGETGEIVWDKGRDFATVRKVLSMPQVNIVKKTEVQTGGFSKESILPKRNSDKLIARKKDWDPKKYGGFDSPTVAYSVLVVAKVEKGKSKKLKSVKELLGITIMERSSFEKNPIDFLEAKGYKEVKKDLIIKLPKYSLFELENGRKRMLASAGELQKGNELALPSKYVNFLYLASHYEKLKGSPEDNEQKQLFVEQHKHYLDEIIEQISEFSKRVILADANLDKVLSAYNKHRDKPIREQAENIIHLFTLTNLGAPAAFKYFDTTIDRKRYTSTKEVLDATLIHQSITGLYETRIDLSQLGGDPIAGSKASPKKKRKVGRAIFKPEELRQALMPTLEALYRQDPESLPFRQPVDPQLLGIPDYFDIVKSPMDLSTIKRKLDTGQYQEPWQYVDDIWLMFNNAWLYNRKTSRVYKYCSKLSEVFEQEIDPVMQSLGYCCGRKLEFSPQTLCCYGKQLCTIPRDATYYSYQNRYHFCEKCFNEIQGESVSLGDDPSQPQTTINKEQFSKRKNDTLDPELFVECTECGRKMHQICVLHHEIIWPAGFVCDGCLKKSARTRKENKFSA

SEQ ID NO: 5 - protein, 1726 aa, Artificial Sequence
  Description of Artificial Sequence: Synthetic polypeptide
MAAFKPNPINYILGLAIGIASVGWAMVEIDEDENPICLIDLGVRVFERAEVPKTGDSLAMARRLARSVRRLTRRRAHRLLRARRLLKREGVLQAADFDENGLIKSLPNTPWQLRAAALDRKLTPLEWSAVLLHLIKHRGYLSQRKNEGETADKELGALLKGVADNAHALQTGDFRTPAELALNKFEKESGHIRNQRGDYSHTFSRKDLQAELILLFEKQKEFGNPHVSGGLKEGIETLLMTQRPALSGDAVQKMLGHCTFEPAEPKAAKNTYTAERFIWLTKLNNLRILEQGSERPLTDTERATLMDEPYRKSKLTYAQARKLLGLEDTAFFKGLRYGKDNAEASTLMEMKAYHAISRALEKEGLKDKKSPLNLSPELQDEIGTAFSLFKTDEDITGRLKDRIQPEILEALLKHISFDKFVQISLKALRRIVPLMEQGKRYDEACAEIYGDHYGKKNTEEKIYLPPIPADEIRNPVVLRALSQARKVINGVVRRYGSPARIHIETAREVGKSFKDRKEIEKRQEENRKDREKAAAKFREYFPNFVGEPKSKDILKLRLYEQQHGKCLYSGKEINLGRLNEKGYVEIAAALPFSRTWDDSFNNKVLVLGSEAQNKGNQTPYEYFNGKDNSREWQEFKARVETSRFPRSKKQRILLQKFDEDGFKERNLNDTRYVNRFLCQFVADRMRLTGKGKKRVFASNGQITNLLRGFWGLRKVRAENDRHHALDAVVVACSTVAMQQKITRFVRYKEMNAFDGKTIDKETGEVLHQKTHFPQPWEFFAQEVMIRVFGKPDGKPEFEEADTPEKLRTLLAEKLSSRPEAVHEYVTPLFVSRAPNRKMSGQGHMETVKSAKRLDEGVSVLRVPLTQLKLKDLEKMVNREREPKLYEALKARLEAHKDDPAKAFAEPFYKYDKAGNRTQQVKAVRVEQVQKTGVWVRNHNGIADNATMVRVDVFEKGDKYYLVPIYSWQVAKGILPDRAVVQGKDEEDWQLIDDSFNFKFSLHPNDLVEVITKKARMFGYFASCHRGTGNINIRIHDLDHKIGKNGILEGIGVKTALSFQKYQIDELGKEIRPCRLKKRPPVRSRADPKKKRKVEASGRAIFKPEELRQALMPTLEALYRQDPESLPFRQPVDPQLLGIPDYFDIVKSPMDLSTIKRKLDTGQYQEPWQYVDDIWLMFNNAWLYNRKTSRVYKYCSKLSEVFEQEIDPVMQSLGYCCGRKLEFSPQTLCCYGKQLCTIPRDATYYSYQNRYHFCEKCFNEIQGESVSLGDDPSQPQTTINKEQFSKRKNDTLDPELFVECTECGRKMHQICVLHHEIIWPAGFVCDGCLKKSARTRKENKFSAKRLPSTRLGTFLENRVNDFLRRQNHPESGEVTVRVVHASDKTVEVKPGMKARFVDSGEMAESFPYRTKALFAFEEIDGVDLCFFGMHVQEYGSDCPPPNQRRVYISYLDSVHFFRPKCLRTAVYHEILIGYLEYVKKLGYTTGHIWACPPSEGDDYIFHCHPPDQKIPKPKRLQEWYKKMLDKAVSERIVHDYKDIFKQATEDRLTSAKELPYFEGDFWPNVLEESIKELEQEEEERKREENTSNESTDVTKGDSKNAKKKNNKKTSKNKSSLSRGNKKKPGMPNVSNDLSQKLYATMEKHKEVFFVIRLIAGPAANSLPPIVDPDPLIPCDLMDGRDAFLTLARDKHLEFSSLRRAQWSTMCMLVELHTQSQDYPYDVPDYAS

SEQ ID NO: 6 - RNA, 100 nt, Artificial Sequence
  Description of Artificial Sequence: Synthetic polynucleotide
ggggccacuagggacaggauguuuuagagcuagaaauagcaaguuaaaauaaggcuaguccguuaucaacuugaaaaaguggcaccgagucggugcuuuu

SEQ ID NO: 7 - RNA, 98 nt, Artificial Sequence
  Description of Artificial Sequence: Synthetic oligonucleotide
ggccacuagggacaggauguuuuagagcuagaaauagcaaguuaaaauaaggcuaguccguuaucaacuugaaaaaguggcaccgagucggugcuuuu

SEQ ID NO: 8 - RNA, 112 nt, Artificial Sequence
  Description of Artificial Sequence: Synthetic polynucleotide
ggggccccuucgggggccacuagggacaggauguuuuagagcuagaaauagcaaguuaaaauaaggcuaguccguuaucaacuugaaaaaguggcaccgagucggugcuuuu

SEQ ID NO: 9 - RNA, 116 nt, Artificial Sequence
  Description of Artificial Sequence: Synthetic polynucleotide
gguaguggccccuucgggggccacuagggacaggauguuuuagagcuagaaauagcaaguuaaaauaaggcuaguccguuaucaacuugaaaaaguggcaccgagucggugcuuuu

SEQ ID NO: 10 - DNA, 1198 bp, Artificial Sequence
  Description of Artificial Sequence: Synthetic polynucleotide
ccaggatcagtgaaacgcaccagacagccgcgtcagagcagctcaggttctgggagagggtagcgcagggtggccactgagaaccgggcaggtcacgcatcccccccttccctcccaccccctgccaagctctccctcccaggatcctctctggctccatcgtaagcaaaccttagaggttctggcaaggagagagatggctccaggaaatgggggtgtgtcaccagataaggaatctgcctaacaggaggtgggggttagacccaatatcaggagactaggaaggaggaggcctaaggatggggcttttctgtcaccaatcctgtccctagtggccccactgtggggtggaggggacagataaaagtacccagaaccagagccacattaaccggccctgggaatataaggtggtcccagctcggggacacaggatccctggaggcagcaaacatgctgtcctgaagtggacataggggcccgggttggaggaagaagactagctgagctctcggacccctggaagatgccatgacagggggctggaagagctagcacagactagagaggtaaggggggtaggggagctgcccaaatgaaaggagtgagaggtgacccggaatccacaggagaacggggtgtccaggcaaagaaagcaagaggatggagaggtggctaaagccagggagacggggtactttggggttgtccagaaaaacggtgatgatgcaggcctacaagaaggggaggcgggacgcaagggagacatccgtcggagaaggccatcctaagaaacgagagatggcacaggccccagaaggagaaggaaaagggaacccagcgagtgaagacggcatggggttgggtgagggaggagagatgcccggagaggacccagacacggggaggatccgctcagaggacatcacgtggtgcagcgccgagaaggaagtgctccggaaagagcatccttgggcagcaacacagcagagagcaaggggaagagggagtggaggaagacggaacctgaaggaggcggcagggaaggatctgggccagccgtagaggtgacccaggccacaagctgcagacagaaagcggcacaggcccaggggagagaatgcaggtcagagaaagcaggacctgcctgggaaggggaaacagtgggccagaggcggcgcagaagccagtagagctc

SEQ ID NO: 11 - DNA, 986 bp, Artificial Sequence
  Description of Artificial Sequence: Synthetic polynucleotide
catgacgtgcagcaagcgcgctgacgcagctaattttatctatgtgcttcgtcatacgtgatgcatatactctctgctagctgactcattcagctgtactcactcgctgttgagtctcatacagcgcgagatcaaatgagtcatccaatcctgtccctagtggcccctatcgtgacactgcactgcagcgtacgcgacagagctagacttcgtttcaatacagactagctactgcgtctgcagagcgctctcttgtcacttacatcgaagtcaacgcgctcgcgttcagagatcttctccaatcctactttcgacaattttcgctctcagcgtttgtgtctgtgcgcgcacacagtctgtgcttcgcttgcaactaacgtagcgcttcagcgcatcgtcaaagagcgaaagagtcacagtgtctgtgttcacgtctctatctttctagttctccaatcctgtcccaaaattgtcgaagacagagtttcgcgaattcgcagcagcgcgatctctgctcactgcaatctctgactgctgcttttaagcaattctcgcagctcagcatgagtacttgcgattacagcagtgctcgccaatcctgtccctagtgattttgcagcgtcagcagagctgatgagatgcagttcagcatcgcagacgagcagcacgaagcgagcatctgtagaaaatcgatcgacgcgcacttgcagagacaccaaaaattgtcgaaagtgaagccttgtctctcgttcgcatcaagacacgctatttctgtctcttaaatgtttcaaaaacacatcatgtcttcttcgtgcgagttcgatgcgcgtgtgcgagaccacgcctgtccctagtggcccctgactctctgtgcattttgagctgcgaaagtaaagatatcgttcattgcagagacagagctagtactagtctcagttcttgcactatgctctcgatgtctctcttagtgattcagcgcatcgtcg

SEQ ID NO: 12 - DNA, 1078 bp, Artificial Sequence
  Description of Artificial Sequence: Synthetic polynucleotide
gacctgcaggcatgcaagcttgggctagcggagagtcagttcgcggtactggaggaggcggcgcaacgtcgccagctgtctgcacaggagaaatccctgctggcgcataaagatgagacgctggagtacaaacgccagctggctgcacttggcgacaaggttacgtatcaggagcgcctgaacgcgctggcgcagcaggcggataaattcgcacagcagcaacgggcaaaacgggccgccattgatgcgaaaagccgggggctgactgaccggcaggcagaacgggaagccacggaacagcgcctgaaggaacagtatggcgataatccgctggcgctgaataacgtcatgtcagagcagaaaaagacctgggcggctgaagaccagcttcgcgggaactggatggcaggcctgaagtccggctggccatgggctgaggccagctgaggtaccgctgaggattgctgaggtgtacagacgctcaagtcagaggtggcgagagctcccggagtggctcacagtcggtggtccggcagtacaatggattaccgtaagacggaaatcactcccgggtatatgaaagagacgaccactgccagggacgaaagtgcaatgcggcatacctcagtggcgtggagtgcaggtatacagattaatccggcagcgtccgtcgttgttgatattgcttatgaaggctccggcagtggcgactggcgtactgacggattcatcgttggggtcggttataaattctgattagccaggtaacacagtgttatgacagcccgccggaaccggtgggcttttttgtggggtgaatatggcagtaaagatttcaggagtcctgaaagacggcacaggaaaaccggtacagaactgcaccattcagctgaaagccagacgtaacagcaccacggtggtggtgaacacggtgggctcagagaatccggatgaagccgggcgttacagcatggatgtggagtacggtcagtacagtgtcatcctgcaggttgacggttttccaccatcgcacgccgggaccatcaccgtgtatgaagattcacaaccggggacgctg

SEQ ID NO: 13 - DNA, 20 bp, Artificial Sequence
  Description of Artificial Sequence: Synthetic oligonucleotide
ttcttcttctgctcggactc

SEQ ID NO: 14 - DNA, 20 bp, Artificial Sequence
  Description of Artificial Sequence: Synthetic oligonucleotide
ttcttcttctgctcggactc

SEQ ID NO: 15 - DNA, 20 bp, Artificial Sequence
  Description of Artificial Sequence: Synthetic oligonucleotide
ttcttcttctgctcggactc

SEQ ID NO: 16 - DNA, 20 bp, Artificial Sequence
  Description of Artificial Sequence: Synthetic oligonucleotide
ttcttcttctgctcggactc

SEQ ID NO: 17 - DNA, 20 bp, Artificial Sequence
  Description of Artificial Sequence: Synthetic oligonucleotide
ttcttcttctgctcggactc

SEQ ID NO: 18 - DNA, 20 bp, Artificial Sequence
  Description of Artificial Sequence: Synthetic oligonucleotide
ttcttcttctgctcggactc

SEQ ID NO: 19 - DNA, 20 bp, Artificial Sequence
  Description of Artificial Sequence: Synthetic oligonucleotide
ttcttcttctgctcggactc

SEQ ID NO: 20 - DNA, 20 bp, Artificial Sequence
  Description of Artificial Sequence: Synthetic oligonucleotide
ttcttcttctgctcggactc

SEQ ID NO: 21 - DNA, 20 bp, Artificial Sequence
  Description of Artificial Sequence: Synthetic oligonucleotide
ttcttcttctgctcggactc

SEQ ID NO: 22 - DNA, 20 bp, Artificial Sequence
  Description of Artificial Sequence: Synthetic oligonucleotide
ttcttcttctgctcggactc

SEQ ID NO: 23 - DNA, 20 bp, Artificial Sequence
  Description of Artificial Sequence: Synthetic oligonucleotide
ttcttcttctgctcggactc

SEQ ID NO: 24 - DNA, 20 bp, Artificial Sequence
  Description of Artificial Sequence: Synthetic oligonucleotide
ttcttcttctgctcggactc

SEQ ID NO: 25 - DNA, 20 bp, Artificial Sequence
  Description of Artificial Sequence: Synthetic oligonucleotide
ttcttcttctgctcggactc

SEQ ID NO: 26 - DNA, 20 bp, Artificial Sequence
  Description of Artificial Sequence: Synthetic oligonucleotide
ttcttcttctgctcggactc

SEQ ID NO: 27 - DNA, 20 bp, Artificial Sequence
  Description of Artificial Sequence: Synthetic oligonucleotide
ttcttcttctgctcggactc

SEQ ID NO: 28 - DNA, 20 bp, Artificial Sequence
  Description of Artificial Sequence: Synthetic oligonucleotide
ttcttcttctgctcggactc

SEQ ID NO: 29 - DNA, 20 bp, Artificial Sequence
  Description of Artificial Sequence: Synthetic oligonucleotide
ttcttcttctgctcggactc

SEQ ID NO: 30 - DNA, 20 bp, Artificial Sequence
  Description of Artificial Sequence: Synthetic oligonucleotide
ttcttcttctgctcggactc

SEQ ID NO: 31 - DNA, 20 bp, Artificial Sequence
  Description of Artificial Sequence: Synthetic oligonucleotide
ttcttcttctgctcggactc

SEQ ID NO: 32 - DNA, 20 bp, Artificial Sequence
  Description of Artificial Sequence: Synthetic oligonucleotide
ttcttcttctgctcggactc

SEQ ID NO: 33 - DNA, 20 bp, Artificial Sequence
  Description of Artificial Sequence: Synthetic oligonucleotide
ccctagtcattggaggtgac

SEQ ID NO: 34 - DNA, 20 bp, Artificial Sequence
  Description of Artificial Sequence: Synthetic oligonucleotide
ccctagtcattggaggtgac

SEQ ID NO: 35 - DNA, 20 bp, Artificial Sequence
  Description of Artificial Sequence: Synthetic oligonucleotide
ccctagtcattggaggtgac

SEQ ID NO: 36 - DNA, 20 bp, Artificial Sequence
  Description of Artificial Sequence: Synthetic oligonucleotide
ccctagtcattggaggtgac

SEQ ID NO: 37 - DNA, 20 bp, Artificial Sequence
  Description of Artificial Sequence: Synthetic oligonucleotide
ccctagtcattggaggtgac

SEQ ID NO: 38 - DNA, 20 bp, Artificial Sequence
  Description of Artificial Sequence: Synthetic oligonucleotide
ccctagtcattggaggtgac

SEQ ID NO: 39 - DNA, 20 bp, Artificial Sequence
  Description of Artificial Sequence: Synthetic oligonucleotide
ccctagtcattggaggtgac

SEQ ID NO: 40 - DNA, 20 bp, Artificial Sequence
  Description of Artificial Sequence: Synthetic oligonucleotide
ccctagtcattggaggtgac

SEQ ID NO: 41 - DNA, 20 bp, Artificial Sequence
  Description of Artificial Sequence: Synthetic oligonucleotide
ccctagtcattggaggtgac

SEQ ID NO: 42 - DNA, 20 bp, Artificial Sequence
  Description of Artificial Sequence: Synthetic oligonucleotide
ccctagtcattggaggtgac

SEQ ID NO: 43 - DNA, 20 bp, Artificial Sequence
  Description of Artificial Sequence: Synthetic oligonucleotide
atggggaggacatcgatgtc

SEQ ID NO: 44 - DNA, 20 bp, Artificial Sequence
  Description of Artificial Sequence: Synthetic oligonucleotide
atggggaggacatcgatgtc

SEQ ID NO: 45 - DNA, 20 bp, Artificial Sequence
  Description of Artificial Sequence: Synthetic oligonucleotide
atggggaggacatcgatgtc

SEQ ID NO: 46 - DNA, 20 bp, Artificial Sequence
  Description of Artificial Sequence: Synthetic oligonucleotide
atggggaggacatcgatgtc

SEQ ID NO: 47 - DNA, 20 bp, Artificial Sequence
  Description of Artificial Sequence: Synthetic oligonucleotide
atggggaggacatcgatgtc

SEQ ID NO: 48 - DNA, 20 bp, Artificial Sequence
  Description of Artificial Sequence: Synthetic oligonucleotide
atggggaggacatcgatgtc

SEQ ID NO: 49 - DNA, 20 bp, Artificial Sequence
  Description of Artificial Sequence: Synthetic oligonucleotide
atggggaggacatcgatgtc

SEQ ID NO: 50 - DNA, 20 bp, Artificial Sequence
  Description of Artificial Sequence: Synthetic oligonucleotide
atggggaggacatcgatgtc

SEQ ID NO: 51 - DNA, 20 bp, Artificial Sequence
  Description of Artificial Sequence: Synthetic oligonucleotide
atggggaggacatcgatgtc

SEQ ID NO: 52 - DNA, 20 bp, Artificial Sequence
  Description of Artificial Sequence: Synthetic oligonucleotide
atggggaggacatcgatgtc

SEQ ID NO: 53 - DNA, 20 bp, Artificial Sequence
  Description of Artificial Sequence: Synthetic oligonucleotide
atcacatcaaccggtggcgc

SEQ ID NO: 54 - DNA, 20 bp, Artificial Sequence
  Description of Artificial Sequence: Synthetic oligonucleotide
atcacatcaaccggtggcgc

SEQ ID NO: 55 - DNA, 20 bp, Artificial Sequence
  Description of Artificial Sequence: Synthetic oligonucleotide
atcacatcaaccggtggcgc

SEQ ID NO: 56 - DNA, 20 bp, Artificial Sequence
  Description of Artificial Sequence: Synthetic oligonucleotide
atcacatcaaccggtggcgc

SEQ ID NO: 57 - DNA, 20 bp, Artificial Sequence
  Description of Artificial Sequence: Synthetic oligonucleotide
atcacatcaaccggtggcgc

SEQ ID NO: 58 - DNA, 20 bp, Artificial Sequence
  Description of Artificial Sequence: Synthetic oligonucleotide
atcacatcaaccggtggcgc

SEQ ID NO: 59 - DNA, 20 bp, Artificial Sequence
  Description of Artificial Sequence: Synthetic oligonucleotide
atcacatcaaccggtggcgc

SEQ ID NO: 60 - DNA, 20 bp, Artificial Sequence
  Description of Artificial Sequence: Synthetic oligonucleotide
atcacatcaaccggtggcgc

SEQ ID NO: 61 - DNA, 20 bp, Artificial Sequence
  Description of Artificial Sequence: Synthetic oligonucleotide
atcacatcaaccggtggcgc

SEQ ID NO: 62 - DNA, 20 bp, Artificial Sequence
  Description of Artificial Sequence: Synthetic oligonucleotide
atcacatcaaccggtggcgc

SEQ ID NO: 63 - DNA, 20 bp, Artificial Sequence
  Description of Artificial Sequence: Synthetic oligonucleotide
gagtttctcatctgtgcccc

SEQ ID NO: 64 - DNA, 20 bp, Artificial Sequence
  Description of Artificial Sequence: Synthetic oligonucleotide
ccagcttctgccgtttgtac

SEQ ID NO: 65 - DNA, 20 bp, Artificial Sequence
  Description of Artificial Sequence: Synthetic oligonucleotide
ccagcttctgccgtttgtac

SEQ ID NO: 66 - DNA, 20 bp, Artificial Sequence
  Description of Artificial Sequence: Synthetic oligonucleotide
ccagcttctgccgtttgtac

SEQ ID NO: 67 - DNA, 20 bp, Artificial Sequence
  Description of Artificial Sequence: Synthetic oligonucleotide
ttcctcctccagcttctgcc

SEQ ID NO: 68 - DNA, 20 bp, Artificial Sequence
  Description of Artificial Sequence: Synthetic oligonucleotide
ttcctcctccagcttctgcc

SEQ ID NO: 69 - DNA, 20 bp, Artificial Sequence
  Description of Artificial Sequence: Synthetic oligonucleotide
ttcctcctccagcttctgcc

SEQ ID NO: 70 - DNA, 20 bp, Artificial Sequence
  Description of Artificial Sequence: Synthetic oligonucleotide
ttcctcctccagcttctgcc

SEQ ID NO: 71 - DNA, 20 bp, Artificial Sequence
  Description of Artificial Sequence: Synthetic oligonucleotide
ttcctcctccagcttctgcc

SEQ ID NO: 72 - DNA, 20 bp, Artificial Sequence
  Description of Artificial Sequence: Synthetic oligonucleotide
ccggttgatgtgatgggagc

SEQ ID NO: 73 - DNA, 20 bp, Artificial Sequence
  Description of Artificial Sequence: Synthetic oligonucleotide
ccggttgatgtgatgggagc

SEQ ID NO: 74 - DNA, 20 bp, Artificial Sequence
  Description of Artificial Sequence: Synthetic oligonucleotide
ccggttgatgtgatgggagc

SEQ ID NO: 75 - DNA, 20 bp, Artificial Sequence
  Description of Artificial Sequence: Synthetic oligonucleotide
ccggttgatgtgatgggagc

SEQ ID NO: 76 - DNA, 20 bp, Artificial Sequence
  Description of Artificial Sequence: Synthetic oligonucleotide
gcagcaagcagcactctgcc

SEQ ID NO: 77 - DNA, 20 bp, Artificial Sequence
  Description of Artificial Sequence: Synthetic oligonucleotide
gcagcaagcagcactctgcc

SEQ ID NO: 78 - DNA, 20 bp, Artificial Sequence
  Description of Artificial Sequence: Synthetic oligonucleotide
gcttgggcccacgcaggggc

SEQ ID NO: 79 - DNA, 20 bp, Artificial Sequence
  Description of Artificial Sequence: Synthetic oligonucleotide
gcttgggcccacgcaggggc

SEQ ID NO: 80 - DNA, 20 bp, Artificial Sequence
  Description of Artificial Sequence: Synthetic oligonucleotide
gcttcgtggcaatgcgccac

SEQ ID NO: 81 - DNA, 20 bp, Artificial Sequence
  Description of Artificial Sequence: Synthetic oligonucleotide
gcttgggcccacgcaggggc

SEQ ID NO: 82 - DNA, 20 bp, Artificial Sequence
  Description of Artificial Sequence: Synthetic oligonucleotide
aagctggactctggccactc

SEQ ID NO: 83 - DNA, 20 bp, Artificial Sequence
  Description of Artificial Sequence: Synthetic oligonucleotide
ttcttcttctgctcggactc

SEQ ID NO: 84 - DNA, 20 bp, Artificial Sequence
  Description of Artificial Sequence: Synthetic oligonucleotide
ttcttcttctgctcggactc

SEQ ID NO: 85 - DNA, 20 bp, Artificial Sequence
  Description of Artificial Sequence: Synthetic oligonucleotide
ttcttcttctgctcggactc

SEQ ID NO: 86 - DNA, 20 bp, Artificial Sequence
  Description of Artificial Sequence: Synthetic oligonucleotide
gagtttctcatctgtgcccc

SEQ ID NO: 87 - DNA, 20 bp, Artificial Sequence
  Description of Artificial Sequence: Synthetic oligonucleotide
ttcctcctccagcttctgcc

SEQ ID NO: 88 - DNA, 20 bp, Artificial Sequence
  Description of Artificial Sequence: Synthetic oligonucleotide
ttcctcctccagcttctgcc

SEQ ID NO: 89 - DNA, 20 bp, Artificial Sequence
  Description of Artificial Sequence: Synthetic oligonucleotide
agcagaagaagaagggctcc

SEQ ID NO: 90 - DNA, 20 bp, Artificial Sequence
  Description of Artificial Sequence: Synthetic oligonucleotide
aagctggactctggccactc

SEQ ID NO: 91 - DNA, 20 bp, Artificial Sequence
  Description of Artificial Sequence: Synthetic oligonucleotide
ccctagtcattggaggtgac

SEQ ID NO: 92 - DNA, 20 bp, Artificial Sequence
  Description of Artificial Sequence: Synthetic oligonucleotide
ccctagtcattggaggtgac

SEQ ID NO: 93 - DNA, 20 bp, Artificial Sequence
  Description of Artificial Sequence: Synthetic oligonucleotide
ccctagtcattggaggtgac

SEQ ID NO: 94 - DNA, 20 bp, Artificial Sequence
  Description of Artificial Sequence: Synthetic oligonucleotide
ccctagtcattggaggtgac

SEQ ID NO: 95 - DNA, 20 bp, Artificial Sequence
  Description of Artificial Sequence: Synthetic oligonucleotide
ccctagtcattggaggtgac

SEQ ID NO: 96 - DNA, 20 bp, Artificial Sequence
  Description of Artificial Sequence: Synthetic oligonucleotide
ccctagtcattggaggtgac

SEQ ID NO: 97 - DNA, 20 bp, Artificial Sequence
  Description of Artificial Sequence: Synthetic oligonucleotide
ccctagtcattggaggtgac

SEQ ID NO: 98 - DNA, 20 bp, Artificial Sequence
  Description of Artificial Sequence: Synthetic oligonucleotide
ccctagtcattggaggtgac

SEQ ID NO: 99 - DNA, 20 bp, Artificial Sequence
  Description of Artificial Sequence: Synthetic oligonucleotide
ccctagtcattggaggtgac

SEQ ID NO: 100 - DNA, 20 bp, Artificial Sequence
  Description of Artificial Sequence: Synthetic oligonucleotide
ccctagtcattggaggtgac

SEQ ID NO: 101 - DNA, 20 bp, Artificial Sequence
  Description of Artificial Sequence: Synthetic oligonucleotide
atggggaggacatcgatgtc

SEQ ID NO: 102 - DNA, 20 bp, Artificial Sequence
  Description of Artificial Sequence: Synthetic oligonucleotide
atggggaggacatcgatgtc

SEQ ID NO: 103 - DNA, 20 bp, Artificial Sequence
  Description of Artificial Sequence: Synthetic oligonucleotide
atggggaggacatcgatgtc

SEQ ID NO: 104 - DNA, 20 bp, Artificial Sequence
  Description of Artificial Sequence: Synthetic oligonucleotide
atggggaggacatcgatgtc

SEQ ID NO: 105 - DNA, 20 bp, Artificial Sequence
  Description of Artificial Sequence: Synthetic oligonucleotide
atggggaggacatcgatgtc

SEQ ID NO: 106 - DNA, 20 bp, Artificial Sequence
  Description of Artificial Sequence: Synthetic oligonucleotide
atggggaggacatcgatgtc

SEQ ID NO: 107 - DNA, 20 bp, Artificial Sequence
  Description of Artificial Sequence: Synthetic oligonucleotide
atggggaggacatcgatgtc

SEQ ID NO: 108 - DNA, 20 bp, Artificial Sequence
  Description of Artificial Sequence: Synthetic oligonucleotide
atggggaggacatcgatgtc

SEQ ID NO: 109 - DNA, 20 bp, Artificial Sequence
  Description of Artificial Sequence: Synthetic oligonucleotide
atggggaggacatcgatgtc

SEQ ID NO: 110 - DNA, 20 bp, Artificial Sequence
  Description of Artificial Sequence: Synthetic oligonucleotide
atggggaggacatcgatgtc

SEQ ID NO: 111 - DNA, 20 bp, Artificial Sequence
  Description of Artificial Sequence: Synthetic oligonucleotide
atcacatcaaccggtggcgc

SEQ ID NO: 112 - DNA, 20 bp, Artificial Sequence
  Description of Artificial Sequence: Synthetic oligonucleotide
atcacatcaaccggtggcgc

SEQ ID NO: 113 - DNA, 20 bp, Artificial Sequence
  Description of Artificial Sequence: Synthetic oligonucleotide
atcacatcaaccggtggcgc

SEQ ID NO: 114 - DNA, 20 bp, Artificial Sequence
  Description of Artificial Sequence: Synthetic oligonucleotide
atcacatcaaccggtggcgc

SEQ ID NO: 115 - DNA, 20 bp, Artificial Sequence
  Description of Artificial Sequence: Synthetic oligonucleotide
atcacatcaaccggtggcgc

SEQ ID NO: 116 - DNA, 20 bp, Artificial Sequence
  Description of Artificial Sequence: Synthetic oligonucleotide
atcacatcaaccggtggcgc

SEQ ID NO: 117 - DNA, 20 bp, Artificial Sequence
  Description of Artificial Sequence: Synthetic oligonucleotide
atcacatcaaccggtggcgc

SEQ ID NO: 118 - DNA, 20 bp, Artificial Sequence
  Description of Artificial Sequence: Synthetic oligonucleotide
atcacatcaaccggtggcgc

SEQ ID NO: 119 - DNA, 20 bp, Artificial Sequence
  Description of Artificial Sequence: Synthetic oligonucleotide
atcacatcaaccggtggcgc

SEQ ID NO: 120 - DNA, 20 bp, Artificial Sequence
  Description of Artificial Sequence: Synthetic oligonucleotide
atcacatcaaccggtggcgc

SEQ ID NO: 121 - DNA, 20 bp, Artificial Sequence
  Description of Artificial Sequence: Synthetic oligonucleotide
gagtttctcatctgtgcccc

SEQ ID NO: 122 - DNA, 20 bp, Artificial Sequence
  Description of Artificial Sequence: Synthetic oligonucleotide
ccagcttctgccgtttgtac

SEQ ID NO: 123 - DNA, 20 bp, Artificial Sequence
  Description of Artificial Sequence: Synthetic oligonucleotide
ccagcttctgccgtttgtac

SEQ ID NO: 124 - DNA, 20 bp, Artificial Sequence
  Description of Artificial Sequence: Synthetic oligonucleotide
ccagcttctgccgtttgtac

SEQ ID NO: 125 - DNA, 20 bp, Artificial Sequence
  Description of Artificial Sequence: Synthetic oligonucleotide
ttcctcctccagcttctgcc

SEQ ID NO: 126 - DNA, 20 bp, Artificial Sequence
  Description of Artificial Sequence: Synthetic oligonucleotide
ttcctcctccagcttctgcc

SEQ ID NO: 127 - DNA, 20 bp, Artificial Sequence
  Description of Artificial Sequence: Synthetic oligonucleotide
ttcctcctccagcttctgcc

SEQ ID NO: 128 - DNA, 20 bp, Artificial Sequence
  Description of Artificial Sequence: Synthetic oligonucleotide
ttcctcctccagcttctgcc

SEQ ID NO: 129 - DNA, 20 bp, Artificial Sequence
  Description of Artificial Sequence: Synthetic oligonucleotide
ttcctcctccagcttctgcc

SEQ ID NO: 130 - DNA, 20 bp, Artificial Sequence
  Description of Artificial Sequence: Synthetic oligonucleotide
ccggttgatgtgatgggagc

SEQ ID NO: 131 - DNA, 20 bp, Artificial Sequence
  Description of Artificial Sequence: Synthetic oligonucleotide
ccggttgatgtgatgggagc

SEQ ID NO: 132 - DNA, 20 bp, Artificial Sequence
  Description of Artificial Sequence: Synthetic oligonucleotide
ccggttgatgtgatgggagc

SEQ ID NO: 133 - DNA, 20 bp, Artificial Sequence
  Description of Artificial Sequence: Synthetic oligonucleotide
ccggttgatgtgatgggagc

SEQ ID NO: 134 - DNA, 20 bp, Artificial Sequence
  Description of Artificial Sequence: Synthetic oligonucleotide
gcagcaagcagcactctgcc

SEQ ID NO: 135 - DNA, 20 bp, Artificial Sequence
  Description of Artificial Sequence: Synthetic oligonucleotide
gcagcaagcagcactctgcc

SEQ ID NO: 136 - DNA, 20 bp, Artificial Sequence
  Description of Artificial Sequence: Synthetic oligonucleotide
gcttgggcccacgcaggggc

SEQ ID NO: 137 - DNA, 20 bp, Artificial Sequence
  Description of Artificial Sequence: Synthetic oligonucleotide
gcttgggcccacgcaggggc

SEQ ID NO: 138 - DNA, 20 bp, Artificial Sequence
  Description of Artificial Sequence: Synthetic oligonucleotide
gcttcgtggcaatgcgccac

SEQ ID NO: 139 - DNA, 20 bp, Artificial Sequence
  Description of Artificial Sequence: Synthetic oligonucleotide
gcttgggcccacgcaggggc

SEQ ID NO: 140 - DNA, 20 bp, Artificial Sequence
  Description of Artificial Sequence: Synthetic oligonucleotide
aagctggactctggccactc

SEQ ID NO: 141 - DNA, 20 bp, Artificial Sequence
  Description of Artificial Sequence: Synthetic oligonucleotide
ttcttcttctgctcggactc

SEQ ID NO: 142 - DNA, 20 bp, Artificial Sequence
  Description of Artificial Sequence: Synthetic oligonucleotide
ttcttcttctgctcggactc

SEQ ID NO: 143 - DNA, 20 bp, Artificial Sequence
  Description of Artificial Sequence: Synthetic oligonucleotide
ttcttcttctgctcggactc

SEQ ID NO: 144 - DNA, 20 bp, Artificial Sequence
  Description of Artificial Sequence: Synthetic oligonucleotide
gagtttctcatctgtgcccc

SEQ ID NO: 145 - DNA, 20 bp, Artificial Sequence
  Description of Artificial Sequence: Synthetic oligonucleotide
ttcctcctccagcttctgcc

SEQ ID NO: 146 - DNA, 20 bp, Artificial Sequence
  Description of Artificial Sequence: Synthetic oligonucleotide
ttcctcctccagcttctgcc

SEQ ID NO: 147 - DNA, 20 bp, Artificial Sequence
  Description of Artificial Sequence: Synthetic oligonucleotide
agcagaagaagaagggctcc

SEQ ID NO: 148 - DNA, 20 bp, Artificial Sequence
  Description of Artificial Sequence: Synthetic oligonucleotide
aagctggactctggccactc

SEQ ID NO: 149 - RNA, 20 nt, Artificial Sequence
  Description of Artificial Sequence: Synthetic oligonucleotide
guguccgagcagaagaagaa

SEQ ID NO: 150 - RNA, 20 nt, Artificial Sequence
  Description of Artificial Sequence: Synthetic oligonucleotide
gacuccgagcagaagaagaa

SEQ ID NO: 151 - RNA, 20 nt, Artificial Sequence
  Description of Artificial Sequence: Synthetic oligonucleotide
gagaccgagcagaagaagaa

SEQ ID NO: 152 - RNA, 20 nt, Artificial Sequence
  Description of Artificial Sequence: Synthetic oligonucleotide
gagugcgagcagaagaagaa

SEQ ID NO: 153 - RNA, 20 nt, Artificial Sequence
  Description of Artificial Sequence: Synthetic oligonucleotide
gagucggagcagaagaagaa

SEQ ID NO: 154 - RNA, 20 nt, Artificial Sequence
  Description of Artificial Sequence: Synthetic oligonucleotide
gagucccagcagaagaagaa

SEQ ID NO: 155 - RNA, 20 nt, Artificial Sequence
  Description of Artificial Sequence: Synthetic oligonucleotide
gaguccgugcagaagaagaa

SEQ ID NO: 156 - RNA, 20 nt, Artificial Sequence
  Description of Artificial Sequence: Synthetic oligonucleotide
gaguccgaccagaagaagaa

SEQ ID NO: 157 - RNA, 20 nt, Artificial Sequence
  Description of Artificial Sequence: Synthetic oligonucleotide
gaguccgaggagaagaagaa

SEQ ID NO: 158 - RNA, 20 nt, Artificial Sequence
  Description of Artificial Sequence: Synthetic oligonucleotide
gaguccgagcugaagaagaa

SEQ ID NO: 159 - RNA, 20 nt, Artificial Sequence
  Description of Artificial Sequence: Synthetic oligonucleotide
guguccgagcagaagaagaa

SEQ ID NO: 160 - RNA, 20 nt, Artificial Sequence
  Description of Artificial Sequence: Synthetic oligonucleotide
gacuccgagcagaagaagaa

SEQ ID NO: 161 - RNA, 20 nt, Artificial Sequence
  Description of Artificial Sequence: Synthetic oligonucleotide
gagaccgagcagaagaagaa

SEQ ID NO: 162 - RNA, 20 nt, Artificial Sequence
  Description of Artificial Sequence: Synthetic oligonucleotide
gagugcgagcagaagaagaa

SEQ ID NO: 163 - RNA, 20 nt, Artificial Sequence
  Description of Artificial Sequence: Synthetic oligonucleotide
gagucggagcagaagaagaa

SEQ ID NO: 164 - RNA, 20 nt, Artificial Sequence
  Description of Artificial Sequence: Synthetic oligonucleotide
gagucccagcagaagaagaa

SEQ ID NO: 165 - RNA, 20 nt, Artificial Sequence
  Description of Artificial Sequence: Synthetic oligonucleotide
gaguccgugcagaagaagaa

SEQ ID NO: 166 - RNA, 20 nt, Artificial Sequence
  Description of Artificial Sequence: Synthetic oligonucleotide
gaguccgaccagaagaagaa

SEQ ID NO: 167 - RNA, 20 nt, Artificial Sequence
  Description of Artificial Sequence: Synthetic oligonucleotide
gaguccgaggagaagaagaa

SEQ ID NO: 168 - RNA, 20 nt, Artificial Sequence
  Description of Artificial Sequence: Synthetic oligonucleotide
gaguccgagcugaagaagaa

SEQ ID NO: 169 - RNA, 20 nt, Artificial Sequence
  Description of Artificial Sequence: Synthetic oligonucleotide
gacaccuccaaugacuaggg

SEQ ID NO: 170 - RNA, 20 nt, Artificial Sequence
  Description of Artificial Sequence: Synthetic oligonucleotide
gugaccuccaaugacuaggg

SEQ ID NO: 171 - RNA, 20 nt, Artificial Sequence
  Description of Artificial Sequence: Synthetic oligonucleotide
gucuccuccaaugacuaggg

SEQ ID NO: 172 - RNA, 20 nt, Artificial Sequence
  Description of Artificial Sequence: Synthetic oligonucleotide
gucagcuccaaugacuaggg

SEQ ID NO: 173 - RNA, 20 nt, Artificial Sequence
  Description of Artificial Sequence: Synthetic oligonucleotide
gucacguccaaugacuaggg

SEQ ID NO: 174 - RNA, 20 nt, Artificial Sequence
  Description of Artificial Sequence: Synthetic oligonucleotide
gucaccaccaaugacuaggg

SEQ ID NO: 175 - RNA, 20 nt, Artificial Sequence
  Description of Artificial Sequence: Synthetic oligonucleotide
gucaccugcaaugacuaggg

SEQ ID NO: 176 - RNA, 20 nt, Artificial Sequence
  Description of Artificial Sequence: Synthetic oligonucleotide
gucaccucgaaugacuaggg

SEQ ID NO: 177 - RNA, 20 nt, Artificial Sequence
  Description of Artificial Sequence: Synthetic oligonucleotide
gucaccuccuaugacuaggg

SEQ ID NO: 178 - RNA, 20 nt, Artificial Sequence
  Description of Artificial Sequence: Synthetic oligonucleotide
gucaccuccauugacuaggg

SEQ ID NO: 179 - RNA, 20 nt, Artificial Sequence
  Description of Artificial Sequence: Synthetic oligonucleotide
gucaucgauguccuccccau

SEQ ID NO: 180 - RNA, 20 nt, Artificial Sequence
  Description of Artificial Sequence: Synthetic oligonucleotide
gagaucgauguccuccccau

SEQ ID NO: 181 - RNA, 20 nt, Artificial Sequence
  Description of Artificial Sequence: Synthetic oligonucleotide
gacuucgauguccuccccau

SEQ ID NO: 182 - RNA, 20 nt, Artificial Sequence
  Description of Artificial Sequence: Synthetic oligonucleotide
gacaacgauguccuccccau

SEQ ID NO: 183 - RNA, 20 nt, Artificial Sequence
  Description of Artificial Sequence: Synthetic oligonucleotide
gacauggauguccuccccau

SEQ ID NO: 184 - RNA, 20 nt, Artificial Sequence
  Description of Artificial Sequence: Synthetic oligonucleotide
gacauccauguccuccccau

SEQ ID NO: 185 - RNA, 20 nt, Artificial Sequence
  Description of Artificial Sequence: Synthetic oligonucleotide
gacaucguuguccuccccau

SEQ ID NO: 186 - RNA, 20 nt, Artificial Sequence
  Description of Artificial Sequence: Synthetic oligonucleotide
gacaucgaaguccuccccau

SEQ ID NO: 187 - RNA, 20 nt, Artificial Sequence
  Description of Artificial Sequence: Synthetic oligonucleotide
gacaucgaucuccuccccau

SEQ ID NO: 188 - RNA, 20 nt, Artificial Sequence
  Description of Artificial Sequence: Synthetic oligonucleotide
gacaucgaugaccuccccau

SEQ ID NO: 189 - RNA, 20 nt, Artificial Sequence
  Description of Artificial Sequence: Synthetic oligonucleotide
gggccaccgguugaugugau

SEQ ID NO: 190 - RNA, 20 nt, Artificial Sequence
  Description of Artificial Sequence: Synthetic oligonucleotide
gccccaccgguugaugugau

SEQ ID NO: 191 - RNA, 20 nt, Artificial Sequence
  Description of Artificial Sequence: Synthetic oligonucleotide
gcggcaccgguugaugugau

SEQ ID NO: 192 - RNA, 20 nt, Artificial Sequence
  Description of Artificial Sequence: Synthetic oligonucleotide
gcgcgaccgguugaugugau

SEQ ID NO: 193 - RNA, 20 nt, Artificial Sequence
  Description of Artificial Sequence: Synthetic oligonucleotide
gcgccuccgguugaugugau

SEQ ID NO: 194 - RNA, 20 nt, Artificial Sequence
  Description of Artificial Sequence: Synthetic oligonucleotide
gcgccagcgguugaugugau

SEQ ID NO: 195 - RNA, 20 nt, Artificial Sequence
  Description of Artificial Sequence: Synthetic oligonucleotide
gcgccacggguugaugugau

SEQ ID NO: 196 - RNA, 20 nt, Artificial Sequence
  Description of Artificial Sequence: Synthetic oligonucleotide
gcgccacccguugaugugau

SEQ ID NO: 197 - RNA, 20 nt, Artificial Sequence
  Description of Artificial Sequence: Synthetic oligonucleotide
gcgccaccgcuugaugugau

SEQ ID NO: 198 - RNA, 20 nt, Artificial Sequence
  Description of Artificial Sequence: Synthetic oligonucleotide
gcgccaccggaugaugugau

SEQ ID NO: 199 - RNA, 20 nt, Artificial Sequence
  Description of Artificial Sequence: Synthetic oligonucleotide
gggccacagaugagaaacuc

SEQ ID NO: 200 - RNA, 20 nt, Artificial Sequence
  Description of Artificial Sequence: Synthetic oligonucleotide
guucaaacggcagaagcugg

SEQ ID NO: 201 - RNA, 20 nt, Artificial Sequence
  Description of Artificial Sequence: Synthetic oligonucleotide
guacuaacggcagaagcugg

SEQ ID NO: 202 - RNA, 20 nt, Artificial Sequence
  Description of Artificial Sequence: Synthetic oligonucleotide
guacaaacgggagaagcugg

SEQ ID NO: 203 - RNA, 20 nt, Artificial Sequence
  Description of Artificial Sequence: Synthetic oligonucleotide
gccagaagcuggaggaggaa

SEQ ID NO: 204 - RNA, 20 nt, Artificial Sequence
  Description of Artificial Sequence: Synthetic oligonucleotide
ggcacaagcuggaggaggaa

SEQ ID NO: 205 - RNA, 20 nt, Artificial Sequence
  Description of Artificial Sequence: Synthetic oligonucleotide
ggcagaaccuggaggaggaa

SEQ ID NO: 206 - RNA, 20 nt, Artificial Sequence
  Description of Artificial Sequence: Synthetic oligonucleotide
ggcagaagcaggaggaggaa

SEQ ID NO: 207 - RNA, 20 nt, Artificial Sequence
  Description of Artificial Sequence: Synthetic oligonucleotide
ggcagaagcucgaggaggaa

SEQ ID NO: 208 - RNA, 20 nt, Artificial Sequence
  Description of Artificial Sequence: Synthetic oligonucleotide
gcacccaucacaucaaccgg

SEQ ID NO: 209 - RNA, 20 nt, Artificial Sequence
  Description of Artificial Sequence: Synthetic oligonucleotide
gcucccuucacaucaaccgg

SEQ ID NO: 210 - RNA, 20 nt, Artificial Sequence
  Description of Artificial Sequence: Synthetic oligonucleotide
gcucccaacacaucaaccgg

SEQ ID NO: 211 - RNA, 20 nt, Artificial Sequence
  Description of Artificial Sequence: Synthetic oligonucleotide
gcucccaucagaucaaccgg

SEQ ID NO: 212 - RNA, 20 nt, Artificial Sequence
  Description of Artificial Sequence: Synthetic oligonucleotide
ggcagugugcugcuugcugc

SEQ ID NO: 213 - RNA, 20 nt, Artificial Sequence
  Description of Artificial Sequence: Synthetic oligonucleotide
ggcagagugcagcuugcugc

SEQ ID NO: 214 - RNA, 20 nt, Artificial Sequence
  Description of Artificial Sequence: Synthetic oligonucleotide
gccccagcgugggcccaagc

SEQ ID NO: 215 - RNA, 20 nt, Artificial Sequence
  Description of Artificial Sequence: Synthetic oligonucleotide
gccccugccugggcccaagc

SEQ ID NO: 216 - RNA, 20 nt, Artificial Sequence
  Description of Artificial Sequence: Synthetic oligonucleotide
guggcccauugccacgaagc

SEQ ID NO: 217 - RNA, 20 nt, Artificial Sequence
  Description of Artificial Sequence: Synthetic oligonucleotide
gccccugcgucggcccaagc

SEQ ID NO: 218 - RNA, 20 nt, Artificial Sequence
  Description of Artificial Sequence: Synthetic oligonucleotide
gaguggccugaguccagcuu

SEQ ID NO: 219 - RNA, 20 nt, Artificial Sequence
  Description of Artificial Sequence: Synthetic oligonucleotide
gagaccgagcagaagaagaa

SEQ ID NO: 220 - RNA, 20 nt, Artificial Sequence
  Description of Artificial Sequence: Synthetic oligonucleotide
gaguccgaggagaagaagaa

SEQ ID NO: 221 - RNA, 20 nt, Artificial Sequence
  Description of Artificial Sequence: Synthetic oligonucleotide
gaguccgagcugaagaagaa

SEQ ID NO: 222 - RNA, 20 nt, Artificial Sequence
  Description of Artificial Sequence: Synthetic oligonucleotide
ggggcacaguugagaaacuc

SEQ ID NO: 223 - RNA, 20 nt, Artificial Sequence
  Description of Artificial Sequence: Synthetic oligonucleotide
ggcagaagguggaggaggaa

SEQ ID NO: 224 - RNA, 20 nt, Artificial Sequence
  Description of Artificial Sequence: Synthetic oligonucleotide
ggcagaagcaggaggaggaa

SEQ ID NO: 225 - RNA, 20 nt, Artificial Sequence
  Description of Artificial Sequence: Synthetic oligonucleotide
ggagcccuuguucuucugcu

SEQ ID NO: 226 - RNA, 20 nt, Artificial Sequence
  Description of Artificial Sequence: Synthetic oligonucleotide
gaguggccugaguccagcuu

SEQ ID NO: 227 - RNA, 20 nt, Artificial Sequence
  Description of Artificial Sequence: Synthetic oligonucleotide
gacaccuccaaugacuaggg

SEQ ID NO: 228 - RNA, 20 nt, Artificial Sequence
  Description of Artificial Sequence: Synthetic oligonucleotide
gugaccuccaaugacuaggg

SEQ ID NO: 229 - RNA, 20 nt, Artificial Sequence
  Description of Artificial Sequence: Synthetic oligonucleotide
gucuccuccaaugacuaggg

SEQ ID NO: 230 - RNA, 20 nt, Artificial Sequence
  Description of Artificial Sequence: Synthetic oligonucleotide
gucagcuccaaugacuaggg

SEQ ID NO: 231 - RNA, 20 nt, Artificial Sequence
  Description of Artificial Sequence: Synthetic oligonucleotide
gucacguccaaugacuaggg

SEQ ID NO: 232 - RNA, 20 nt, Artificial Sequence
  Description of Artificial Sequence: Synthetic oligonucleotide
gucaccaccaaugacuaggg

SEQ ID NO: 233 - RNA, 20 nt, Artificial Sequence
  Description of Artificial Sequence: Synthetic oligonucleotide
gucaccugcaaugacuaggg

SEQ ID NO: 234 - RNA, 20 nt, Artificial Sequence
  Description of Artificial Sequence: Synthetic oligonucleotide
gucaccucgaaugacuaggg

SEQ ID NO: 235 - RNA, 20 nt, Artificial Sequence
  Description of Artificial Sequence: Synthetic oligonucleotide
gucaccuccuaugacuaggg

SEQ ID NO: 236 - RNA, 20 nt, Artificial Sequence
  Description of Artificial Sequence: Synthetic oligonucleotide
gucaccuccauugacuaggg

SEQ ID NO: 237 - RNA, 20 nt, Artificial Sequence
  Description of Artificial Sequence: Synthetic oligonucleotide
gucaucgauguccuccccau

SEQ ID NO: 238 - RNA, 20 nt, Artificial Sequence
  Description of Artificial Sequence: Synthetic oligonucleotide
gagaucgauguccuccccau

SEQ ID NO: 239 - RNA, 20 nt, Artificial Sequence
  Description of Artificial Sequence: Synthetic oligonucleotide
gacuucgauguccuccccau

SEQ ID NO: 240 - RNA, 20 nt, Artificial Sequence
  Description of Artificial Sequence: Synthetic oligonucleotide
gacaacgauguccuccccau

SEQ ID NO: 241 - RNA, 20 nt, Artificial Sequence
  Description of Artificial Sequence: Synthetic oligonucleotide
gacauggauguccuccccau

SEQ ID NO: 242 - RNA, 20 nt, Artificial Sequence
  Description of Artificial Sequence: Synthetic oligonucleotide
gacauccauguccuccccau

SEQ ID NO: 243 - RNA, 20 nt, Artificial Sequence
  Description of Artificial Sequence: Synthetic oligonucleotide
gacaucguuguccuccccau

SEQ ID NO: 244 - RNA, 20 nt, Artificial Sequence
  Description of Artificial Sequence: Synthetic oligonucleotide
gacaucgaaguccuccccau

SEQ ID NO: 245 - RNA, 20 nt, Artificial Sequence
  Description of Artificial Sequence: Synthetic oligonucleotide
gacaucgaucuccuccccau

SEQ ID NO: 246 - RNA, 20 nt, Artificial Sequence
  Description of Artificial Sequence: Synthetic oligonucleotide
gacaucgaugaccuccccau

SEQ ID NO: 247 - RNA, 20 nt, Artificial Sequence
  Description of Artificial Sequence: Synthetic oligonucleotide
gggccaccgguugaugugau

SEQ ID NO: 248 - RNA, 20 nt, Artificial Sequence
  Description of Artificial Sequence: Synthetic oligonucleotide
gccccaccgguugaugugau

SEQ ID NO: 249 - RNA, 20 nt, Artificial Sequence
  Description of Artificial Sequence: Synthetic oligonucleotide
gcggcaccgguugaugugau

SEQ ID NO: 250 - RNA, 20 nt, Artificial Sequence
  Description of Artificial Sequence: Synthetic oligonucleotide
gcgcgaccgguugaugugau

SEQ ID NO: 251 - RNA, 20 nt, Artificial Sequence
  Description of Artificial Sequence: Synthetic oligonucleotide
gcgccuccgguugaugugau

SEQ ID NO: 252 - RNA, 20 nt, Artificial Sequence
  Description of Artificial Sequence: Synthetic oligonucleotide
gcgccagcgguugaugugau

SEQ ID NO: 253 - RNA, 20 nt, Artificial Sequence
  Description of Artificial Sequence: Synthetic oligonucleotide
gcgccacggguugaugugau

SEQ ID NO: 254 - RNA, 20 nt, Artificial Sequence
  Description of Artificial Sequence: Synthetic oligonucleotide
gcgccacccguugaugugau

SEQ ID NO: 255 - RNA, 20 nt, Artificial Sequence
  Description of Artificial Sequence: Synthetic oligonucleotide
gcgccaccgcuugaugugau

SEQ ID NO: 256 - RNA, 20 nt, Artificial Sequence
  Description of Artificial Sequence: Synthetic oligonucleotide
gcgccaccggaugaugugau

SEQ ID NO: 257 - RNA, 20 nt, Artificial Sequence
  Description of Artificial Sequence: Synthetic oligonucleotide
gggccacagaugagaaacuc

SEQ ID NO: 258 - RNA, 20 nt, Artificial Sequence
  Description of Artificial Sequence: Synthetic oligonucleotide
guucaaacggcagaagcugg

SEQ ID NO: 259 - RNA, 20 nt, Artificial Sequence
  Description of Artificial Sequence: Synthetic oligonucleotide
guacuaacggcagaagcugg

SEQ ID NO: 260 - RNA, 20 nt, Artificial Sequence
  Description of Artificial Sequence: Synthetic oligonucleotide
guacaaacgggagaagcugg

SEQ ID NO: 261 - RNA, 20 nt, Artificial Sequence
  Description of Artificial Sequence: Synthetic oligonucleotide
gccagaagcuggaggaggaa

SEQ ID NO: 262 - RNA, 20 nt, Artificial Sequence
  Description of Artificial Sequence: Synthetic oligonucleotide
ggcacaagcuggaggaggaa

SEQ ID NO: 263 - RNA, 20 nt, Artificial Sequence
  Description of Artificial Sequence: Synthetic oligonucleotide
ggcagaaccuggaggaggaa

SEQ ID NO: 264 - RNA, 20 nt, Artificial Sequence
  Description of Artificial Sequence: Synthetic oligonucleotide
ggcagaagcaggaggaggaa

SEQ ID NO: 265 - RNA, 20 nt, Artificial Sequence
  Description of Artificial Sequence: Synthetic oligonucleotide
ggcagaagcucgaggaggaa

SEQ ID NO: 266 - RNA, 20 nt, Artificial Sequence
  Description of Artificial Sequence: Synthetic oligonucleotide
gcacccaucacaucaaccgg

SEQ ID NO: 267 - RNA, 20 nt, Artificial Sequence
  Description of Artificial Sequence: Synthetic oligonucleotide
gcucccuucacaucaaccgg

SEQ ID NO: 268 - RNA, 20 nt, Artificial Sequence
  Description of Artificial Sequence: Synthetic oligonucleotide
gcucccaacacaucaaccgg

SEQ ID NO: 269 - RNA, 20 nt, Artificial Sequence
  Description of Artificial Sequence: Synthetic oligonucleotide
gcucccaucagaucaaccgg

SEQ ID NO: 270 - RNA, 20 nt, Artificial Sequence
  Description of Artificial Sequence: Synthetic oligonucleotide
ggcagugugcugcuugcugc

SEQ ID NO: 271 - RNA, 20 nt, Artificial Sequence
  Description of Artificial Sequence: Synthetic oligonucleotide
ggcagagugcagcuugcugc

SEQ ID NO: 272 - RNA, 20 nt, Artificial Sequence
  Description of Artificial Sequence: Synthetic oligonucleotide
gccccagcgugggcccaagc

SEQ ID NO: 273 - RNA, 20 nt, Artificial Sequence
  Description of Artificial Sequence: Synthetic oligonucleotide
gccccugccugggcccaagc

SEQ ID NO: 274 - RNA, 20 nt, Artificial Sequence
  Description of Artificial Sequence: Synthetic oligonucleotide
guggcccauugccacgaagc

SEQ ID NO: 275 - RNA, 20 nt, Artificial Sequence
  Description of Artificial Sequence: Synthetic oligonucleotide
gccccugcgucggcccaagc

SEQ ID NO: 276 - RNA, 20 nt, Artificial Sequence
  Description of Artificial Sequence: Synthetic oligonucleotide
gaguggccugaguccagcuu

SEQ ID NO: 277 - RNA, 20 nt, Artificial Sequence
  Description of Artificial Sequence: Synthetic oligonucleotide
gagaccgagcagaagaagaa

SEQ ID NO: 278 - RNA, 20 nt, Artificial Sequence
  Description of Artificial Sequence: Synthetic oligonucleotide
gaguccgaggagaagaagaa

SEQ ID NO: 279 - RNA, 20 nt, Artificial Sequence
  Description of Artificial Sequence: Synthetic oligonucleotide
gaguccgagcugaagaagaa

SEQ ID NO: 280 - RNA, 20 nt, Artificial Sequence
  Description of Artificial Sequence: Synthetic oligonucleotide
ggggcacaguugagaaacuc

SEQ ID NO: 281 - RNA, 20 nt, Artificial Sequence
  Description of Artificial Sequence: Synthetic oligonucleotide
ggcagaagguggaggaggaa

SEQ ID NO: 282 - RNA, 20 nt, Artificial Sequence
  Description of Artificial Sequence: Synthetic oligonucleotide
ggcagaagcaggaggaggaa

SEQ ID NO: 283 - RNA, 20 nt, Artificial Sequence
  Description of Artificial Sequence: Synthetic oligonucleotide
ggagcccuuguucuucugcu

SEQ ID NO: 284 - RNA, 20 nt, Artificial Sequence
  Description of Artificial Sequence: Synthetic oligonucleotide
gaguggccugaguccagcuu

SEQ ID NO: 285 - DNA, 24 bp, Artificial Sequence
  Description of Artificial Sequence: Synthetic oligonucleotide
gagttcctactcagactgttactc

SEQ ID NO: 286 - DNA, 26 bp, Artificial Sequence
  Description of Artificial Sequence: Synthetic oligonucleotide
gtgagttcctactcagactgttactc

SEQ ID NO: 287 - DNA, 28 bp, Artificial Sequence
  Description of Artificial Sequence: Synthetic oligonucleotide
gtctgagttcctactcagactgttactc

SEQ ID NO: 288 - DNA, 24 bp, Artificial Sequence
  Description of Artificial Sequence: Synthetic oligonucleotide
gtattcgtactcagactgttactc

SEQ ID NO: 289 - DNA, 26 bp, Artificial Sequence
  Description of Artificial Sequence: Synthetic oligonucleotide
gagtattcgtactcagactgttactc

SEQ ID NO: 290 - DNA, 25 bp, Artificial Sequence
  Description of Artificial Sequence: Synthetic oligonucleotide
gacttcggtccgagcagaagaagaa

SEQ ID NO: 291 - DNA, 26 bp, Artificial Sequence
  Description of Artificial Sequence: Synthetic oligonucleotide
ggacttcggtccgagcagaagaagaa

SEQ ID NO: 292 - DNA, 28 bp, Artificial Sequence
  Description of Artificial Sequence: Synthetic oligonucleotide
gcggacttcggtccgagcagaagaagaa

SEQ ID NO: 293 - DNA, 24 bp, Artificial Sequence
  Description of Artificial Sequence: Synthetic oligonucleotide
gcgggagtccgagcagaagaagaa

SEQ ID NO: 294 - DNA, 25 bp, Artificial Sequence
  Description of Artificial Sequence: Synthetic oligonucleotide
gtcgggagtccgagcagaagaagaa

SEQ ID NO: 295 - DNA, 26 bp, Artificial Sequence
  Description of Artificial Sequence: Synthetic oligonucleotide
gctcgggagtccgagcagaagaagaa

SEQ ID NO: 296 - DNA, 30 bp, Artificial Sequence
  Description of Artificial Sequence: Synthetic oligonucleotide
gttcacttcggggtggggggagtttgctcc

SEQ ID NO: 297 - DNA, 29 bp, Artificial Sequence
  Description of Artificial Sequence: Synthetic oligonucleotide
gttcattcggggtggggggagtttgctcc

SEQ ID NO: 298 - DNA, 28 bp, Artificial Sequence
  Description of Artificial Sequence: Synthetic oligonucleotide
gtccttcggggtggggggagtttgctcc

SEQ ID NO: 299 - DNA, 30 bp, Artificial Sequence
  Description of Artificial Sequence: Synthetic oligonucleotide
gcttccttcggggtggggggagtttgctcc

SEQ ID NO: 300 - DNA, 30 bp, Artificial Sequence
  Description of Artificial Sequence: Synthetic oligonucleotide
gtttccttcggggtggggggagtttgctcc

SEQ ID NO: 301 - DNA, 29 bp, Artificial Sequence
  Description of Artificial Sequence: Synthetic oligonucleotide
gctccttcggggtggggggagtttgctcc

SEQ ID NO: 302 - DNA, 30 bp, Artificial Sequence
  Description of Artificial Sequence: Synthetic oligonucleotide
gcccacttcggggtggggggagtttgctcc

SEQ ID NO: 303 - DNA, 29 bp, Artificial Sequence
  Description of Artificial Sequence: Synthetic oligonucleotide
gcccattcggggtggggggagtttgctcc

SEQ ID NO: 304 - DNA, 29 bp, Artificial Sequence
  Description of Artificial Sequence: Synthetic oligonucleotide
gccccttcggggtggggggagtttgctcc

SEQ ID NO: 305 - DNA, 30 bp, Artificial Sequence
  Description of Artificial Sequence: Synthetic oligonucleotide
gcatccttcggtgtggggggagtttgctcc

SEQ ID NO: 306 - DNA, 25 bp, Artificial Sequence
  Description of Artificial Sequence: Synthetic oligonucleotide
gccccgggtggggggagtttgctcc

SEQ ID NO: 307 - DNA, 24 bp, Artificial Sequence
  Description of Artificial Sequence: Synthetic oligonucleotide
gcccgggtggggggagtttgctcc

SEQ ID NO: 308 - DNA, 23 bp, Artificial Sequence
  Description of Artificial Sequence: Synthetic oligonucleotide
gccgggtggggggagtttgctcc

SEQ ID NO: 309 - DNA, 29 bp, Artificial Sequence
  Description of Artificial Sequence: Synthetic oligonucleotide
gcacgttcgggtgagtgagtgtgtgcgtg

SEQ ID NO: 310 - DNA, 29 bp, Artificial Sequence
  Description of Artificial Sequence: Synthetic oligonucleotide
gtacgttcgggtgagtgagtgtgtgcgtg

SEQ ID NO: 311 - DNA, 29 bp, Artificial Sequence
  Description of Artificial Sequence: Synthetic oligonucleotide
gcatgttcgggtgagtgagtgtgtgcgtg

SEQ ID NO: 312 - DNA, 29 bp, Artificial Sequence
  Description of Artificial Sequence: Synthetic oligonucleotide
gtatgttcgggtgagtgagtgtgtgcgtg

SEQ ID NO: 313 - DNA, 29 bp, Artificial Sequence
  Description of Artificial Sequence: Synthetic oligonucleotide
gcgcgttcgggtgagtgagtgtgtgcgtg

SEQ ID NO: 314 - DNA, 29 bp, Artificial Sequence
  Description of Artificial Sequence: Synthetic oligonucleotide
gcgtgttcgggtgagtgagtgtgtgcgtg

SEQ ID NO: 315 - DNA, 28 bp, Artificial Sequence
  Description of Artificial Sequence: Synthetic oligonucleotide
gtaggttcgcctactcagactgttactc

SEQ ID NO: 316 - DNA, 21 bp, Artificial Sequence
  Description of Artificial Sequence: Synthetic oligonucleotide
ggcctccccaaagcctggcca

SEQ ID NO: 317 - DNA, 21 bp, Artificial Sequence
  Description of Artificial Sequence: Synthetic oligonucleotide
gacctccccatagcctggcca

SEQ ID NO: 318 - DNA, 6 bp, Artificial Sequence
  Description of Artificial Sequence: Synthetic oligonucleotide
gggagt

SEQ ID NO: 319 - DNA, 6 bp, Artificial Sequence
  Description of Artificial Sequence: Synthetic oligonucleotide
gggagg

SEQ ID NO: 320 - DNA, 27 bp, Artificial Sequence
  Description of Artificial Sequence: Synthetic oligonucleotide
tttcctgatggtccatgtctgttactc

SEQ ID NO: 321 - DNA, 27 bp, Artificial Sequence
  Description of Artificial Sequence: Synthetic oligonucleotide
tttcgtgatggtccatgtctgttactc

SEQ ID NO: 322 - DNA, 27 bp, Artificial Sequence
  Description of Artificial Sequence: Synthetic oligonucleotide
tttccagttggtccatgtctgttactc

SEQ ID NO: 323 - DNA, 27 bp, Artificial Sequence
  Description of Artificial Sequence: Synthetic oligonucleotide
tttcctgatggtccatgtctgttactg

SEQ ID NO: 324 - DNA, 20 bp, Artificial Sequence
  Description of Artificial Sequence: Synthetic primer
ctgggactcaggcgggtcac

SEQ ID NO: 325 - DNA, 25 bp, Artificial Sequence
  Description of Artificial Sequence: Synthetic primer
cctcacacaacagcttcatgtcagc

SEQ ID NO: 326 - DNA, 20 bp, Artificial Sequence
  Description of Artificial Sequence: Synthetic oligonucleotide
ctgatggtgcatgtctgtta

SEQ ID NO: 327 - DNA, 17 bp, Artificial Sequence
  Description of Artificial Sequence: Synthetic oligonucleotide
ctgatggtgcatgtctg

SEQ ID NO: 328 - DNA, 32 bp, Artificial Sequence
  Description of Artificial Sequence: Synthetic oligonucleotide
ctgatggtgcatgtctgttaagacatgcacca

SEQ ID NO: 329 - DNA, 26 bp, Artificial Sequence
  Description of Artificial Sequence: Synthetic oligonucleotide
ctgatggtgcatgtctgcatgcacca

SEQ ID NO: 330 - DNA, 28 bp, Unknown
  Description of Unknown: DNMT1 oligonucleotide
tttcctgatgggtccatgtctgttactc

SEQ ID NO: 331 - DNA, 20 bp, Artificial Sequence
  Description of Artificial Sequence: Synthetic oligonucleotide
ctgatggtgcatgtctgtta

SEQ ID NO: 332 - DNA, 17 bp, Artificial Sequence
  Description of Artificial Sequence: Synthetic oligonucleotide
ctgatggtgcatgtctg

SEQ ID NO: 333 - DNA, 32 bp, Artificial Sequence; identical to SEQ ID NO: 328
  Description of Artificial Sequence: Synthetic oligonucleotide

SEQ ID NO: 334 - DNA, 26 bp, Artificial Sequence
  Description of Artificial Sequence: Synthetic oligonucleotide
ctgatggtgcatgtctgcatgcacca

SEQ ID NO: 335 - DNA, 32 bp, Artificial Sequence
  Description of Artificial Sequence: Synthetic oligonucleotide
gtgagtaggttcgcctactcagactgttactc

SEQ ID NO: 336 - DNA, 20 bp, Artificial Sequence
  Description of Artificial Sequence: Synthetic oligonucleotide
atcctgtccctagtggcccc

SEQ ID NO: 337 - DNA, 20 bp, Artificial Sequence
  Description of Artificial Sequence: Synthetic oligonucleotide
ggggccactagggacaggat

SEQ ID NO: 338 - RNA, 20 nt, Artificial Sequence
  Description of Artificial Sequence: Synthetic oligonucleotide
ggggccacuagggacaggau

SEQ ID NO: 339 - RNA, 18 nt, Artificial Sequence
  Description of Artificial Sequence: Synthetic oligonucleotide
ggccacuagggacaggau

SEQ ID NO: 340 - DNA, 20 bp, Unknown
  Description of Unknown: VEGFA1 target site oligonucleotide
gggtggggggagtttgctcc

SEQ ID NO: 341 - DNA, 20 bp, Unknown
  Description of Unknown: VEGFA1 off-target site oligonucleotide
ggatggagggagtttgctcc

SEQ ID NO: 342 - protein, 6 aa, Artificial Sequence
  Description of Artificial Sequence: Synthetic 6xHis tag
HHHHHH

SEQ ID NO: 343 - DNA, 20 bp, Artificial Sequence
  Description of Artificial Sequence: Synthetic primer
  5'-Biotinylation
ccaggatcagtgaaacgcac

SEQ ID NO: 344 - DNA, 20 bp, Artificial Sequence
  Description of Artificial Sequence: Synthetic primer
gagctctactggcttctgcg

SEQ ID NO: 345 - DNA, 17 bp, Artificial Sequence
  Description of Artificial Sequence: Synthetic primer
  5'-Biotinylation
catgacgtgcagcaagc

SEQ ID NO: 346 - DNA, 17 bp, Artificial Sequence
  Description of Artificial Sequence: Synthetic primer
cgacgatgcgctgaatc

SEQ ID NO: 347 - DNA, 23 bp, Artificial Sequence
  Description of Artificial Sequence: Synthetic primer
  5'-Biotinylation
gacctgcaggcatgcaagcttgg

SEQ ID NO: 348 - DNA, 22 bp, Artificial Sequence
  Description of Artificial Sequence: Synthetic primer
cagcgtccccggttgtgaatct